European Patent Application EP 4 129 344 A1, published February 8, 2023. Title: Immunity-inducing agent comprising polynucleotide-peptide conjugate and pharmaceutical composition comprising same. Applicant: THE UNIVERSITY OF KITAKYUSHU DAIICHI SANKYO COMPANY, LIMITED. The sequence listing filed with the application follows.

SEQUENCE LISTING (54 sequences)

SEQ ID NO: 1 - DNA, 20 bp, Artificial Sequence
  K3
atcgactctcgagcgttctc

SEQ ID NO: 2 - DNA, 20 bp, Artificial Sequence
  K3-20(b)
gagcgttctcgagcgttctc

SEQ ID NO: 3 - DNA, 21 bp, Artificial Sequence
  K3-21
cgagcgttctcgagcgttctc

SEQ ID NO: 4 - DNA, 24 bp, Artificial Sequence
  K3-24
tctcgagcgttctcgagcgttctc

SEQ ID NO: 5 - DNA, 27 bp, Artificial Sequence
  K3-27
gactctcgagcgttctcgagcgttctc

SEQ ID NO: 6 - DNA, 30 bp, Artificial Sequence
  K3-30(a)
gagcgttctcatcgactctcgagcgttctc

SEQ ID NO: 7 - DNA, 30 bp, Artificial Sequence
  K3-30(b)
atcgactctcgagcgttctcgagcgttctc

SEQ ID NO: 8 - DNA, 40 bp, Artificial Sequence
  K3-40
atcgactctcgagcgttctcatcgactctcgagcgttctc

SEQ ID NO: 9 - DNA, 30 bp, Artificial Sequence
  K3-30(c)
ctcagcgttctcagcgttctcagcgttctc

SEQ ID NO: 10 - DNA, 30 bp, Artificial Sequence
  K3-30(d)
tttagcgtttttagcgtttttagcgttttt

SEQ ID NO: 11 - DNA, 30 bp, Artificial Sequence
  K3-30(e)
ttagcgtttagcgtttagcgtttagcgttt

SEQ ID NO: 12 - DNA, 30 bp, Artificial Sequence
  K3-30(f)
ttagcgttcagcgttcagcgttcagcgttt

SEQ ID NO: 13 - DNA, 26 bp, Artificial Sequence
  K3-26(a)
tcagcgtttcagcgtttcagcgtttc

SEQ ID NO: 14 - DNA, 26 bp, Artificial Sequence
  K3-26(b)
ttagcgttttagcgttttagcgtttt

SEQ ID NO: 15 - DNA, 20 bp, Artificial Sequence
  ODN1668
tccatgacgttcctgatgct

SEQ ID NO: 16 - DNA, 30 bp, Artificial Sequence
  ODN1668-30
tgacgttccttccatgacgttcctgatgct

SEQ ID NO: 17 - DNA, 40 bp, Artificial Sequence
  ODN1668-40
tccatgacgttcctgatgcttccatgacgttcctgatgct

SEQ ID NO: 18 - DNA, 20 bp, Artificial Sequence
  ODN1826
tccatgacgttcctgacgtt

SEQ ID NO: 19 - DNA, 30 bp, Artificial Sequence
  ODN1826-30
tgacgttccttccatgacgttcctgacgtt

SEQ ID NO: 20 - DNA, 40 bp, Artificial Sequence
  ODN1826-40
tccatgacgttcctgacgtttccatgacgttcctgacgtt

SEQ ID NO: 21 - DNA, 24 bp, Artificial Sequence
  ODN2006
tcgtcgttttgtcgttttgtcgtt

SEQ ID NO: 22 - DNA, 30 bp, Artificial Sequence
  ODN2006-30
gtcgtttcgtcgttttgtcgttttgtcgtt

SEQ ID NO: 23 - DNA, 40 bp, Artificial Sequence
  ODN2006-40
tcgtcgttttgtcgtttcgtcgttttgtcgttttgtcgtt

SEQ ID NO: 24 - DNA, 23 bp, Artificial Sequence
  ODN684
tcgacgttcgtcgttcgtcgttc

SEQ ID NO: 25 - DNA, 30 bp, Artificial Sequence
  ODN684-30
tcgtcgttcgacgttcgtcgttcgtcgttc

SEQ ID NO: 26 - DNA, 40 bp, Artificial Sequence
  ODN684-40
gttcgtcgtttcgtcgttcgacgttcgtcgttcgtcgttc

SEQ ID NO: 27 - DNA, 26 bp, Artificial Sequence
  ODN D-SL01
tcgcgacgttcgcccgacgttcggta

SEQ ID NO: 28 - DNA, 35 bp, Artificial Sequence
  ODN D-SL01-35
tcgcgacgttcgcgacgttcgcccgacgttcggta

SEQ ID NO: 29 - DNA, 30 bp, Artificial Sequence
  C-CpG_1
tcgaacgttcgaacgttcgaacgttcgaat

SEQ ID NO: 30 - protein, 9 aa, Artificial Sequence
  C-OVA8
CSIINFEKL

SEQ ID NO: 31 - protein, 10 aa, Artificial Sequence
  C-TRP2-9
CSVYDFFVWL

SEQ ID NO: 32 - protein, 9 aa, Artificial Sequence
  C-TRP2-8
CVYDFFVWL

SEQ ID NO: 33 - protein, 10 aa, Artificial Sequence
  C-gp100-9
CKVPRNQDWL

SEQ ID NO: 34 - protein, 9 aa, Artificial Sequence
  C-gp100-8
CVPRNQDWL

SEQ ID NO: 35 - protein, 11 aa, Artificial Sequence
  CM-TRP2-9
CMSVYDFFVWL

SEQ ID NO: 36 - protein, 14 aa, Artificial Sequence
  C-TRP2-13
CFANASVYDFFVWL

SEQ ID NO: 37 - protein, 12 aa, Artificial Sequence
  C-TRP2-11
CNASVYDFFVWL

SEQ ID NO: 38 - protein, 18 aa, Artificial Sequence
  C-OVA2-17
CISQAVHAAHAEINEAGR

SEQ ID NO: 39 - protein, 15 aa, Artificial Sequence
  C-OVA2-14
CSQAVHAAHAEINEA

SEQ ID NO: 40 - protein, 12 aa, Artificial Sequence
  C-OVA2-11
CAVHAAHAEINE

SEQ ID NO: 41 - protein, 8 aa, Artificial Sequence
  OVA peptide 1
SIINFEKL

SEQ ID NO: 42 - protein, 17 aa, Artificial Sequence
  OVA peptide 2
ISQAVHAAHAEINEAGR

SEQ ID NO: 43 - DNA, 22 bp, Artificial Sequence
  1018ISS
tgactgtgaacgttcgagatga

SEQ ID NO: 44 - DNA, 30 bp, Artificial Sequence
  1018ISS_30
tgaacgttcgactgtgaacgttcgagatga

SEQ ID NO: 45 - DNA, 40 bp, Artificial Sequence
  1018ISS_40
tgaacgttcgtgaacgttcgactgtgaacgttcgagatga

SEQ ID NO: 46 - protein, 8 aa, Artificial Sequence
  C-OVA7
CIINFEKL

SEQ ID NO: 47 - DNA, 16 bp, Artificial Sequence
  compK3
gagaacgctcgagagt

SEQ ID NO: 48 - protein, 15 aa, Artificial Sequence
  C-OVA2-14
CSQAVHAAHAEINEA

SEQ ID NO: 49 - protein, 18 aa, Artificial Sequence
  C-OVA2-17
CISQAVHAAHAEINEAGR

SEQ ID NO: 50 - protein, 18 aa, Artificial Sequence
  OVA2-17-C
ISQAVHAAHAEINEAGRC

SEQ ID NO: 51 - protein, 17 aa, Artificial Sequence
  C-OVA2-16
CSQAVHAAHAEINEAGR

SEQ ID NO: 52 - protein, 9 aa, Artificial Sequence
  dC-mTRP2pep8
  X (1)..(1): D-cysteine
XVYDFFVWL

SEQ ID NO: 53 - protein, 9 aa, Artificial Sequence
  homoC-mTRP2pep8
  X (1)..(1): L-homocysteine
XVYDFFVWL

SEQ ID NO: 54 - protein, 9 aa, Artificial Sequence
  Pen-mTRP2pep8
  X (1)..(1): L-penicillamine
XVYDFFVWL